European Patent Application EP 4 317 439 A1, published February 7, 2024. Title: Chimeric antigen receptor that recognizes CCR8 as an antigen. Applicant: SHIONOGI & CO., LTD. OSAKA UNIVERSITY. The sequence listing filed with the application follows.

SEQUENCE LISTING (62 sequences)

SEQ ID NO: 1 - protein, 21 aa, Homo sapiens
MALPVTALLLPLALLLHAARP

SEQ ID NO: 2 - protein, 15 aa, Artificial Sequence
  G4S peptide linker
GGGGSGGGGSGGGGS

SEQ ID NO: 3 - protein, 12 aa, Artificial Sequence
  Linker and Flag epitope
ANASDYKDDDDK

SEQ ID NO: 4 - protein, 45 aa, Homo sapiens
TTTPAPRPPTPAPTIASQPLSLRPEACRPAAGGAVHTRGLDFACD

SEQ ID NO: 5 - protein, 24 aa, Homo sapiens
IYIWAPLAGTCGVLLLSLVITLYC

SEQ ID NO: 6 - protein, 27 aa, Homo sapiens
FWVLVVVGGVLACYSLLVTVAFIIFWV

SEQ ID NO: 7 - protein, 41 aa, Homo sapiens
RSKRSRLLHSDYMNMTPRRPGPTRKHYQPYAPPRDFAAYRS

SEQ ID NO: 8 - protein, 42 aa, Homo sapiens
KRGRKKLLYIFKQPFMRPVQTTQEEDGCSCRFPEEEEGGCEL

SEQ ID NO: 9 - protein, 120 aa, Homo sapiens
WRRKRKEKQSETSPKEFLTIYEDVKDLKTRRNHEQEQTFPGGGSTIYSMIQSQSSAPTSQEPAYTLYSLIQPSRKSGSRKRNHSPSFNSTIYEVIGKSQPKAQNPARLSRKELENFDVYS

SEQ ID NO: 10 - protein, 113 aa, Homo sapiens
RVKFSRSADAPAYQQGQNQLYNELNLGRREEYDVLDKRRGRDPEMGGKPQRRKNPQEGLYNELQKDKMAEAYSEIGMKGERRRGKGHDGLYQGLSTATKDTYDALHMQALPPR

SEQ ID NO: 11 - protein, 24 aa, Homo sapiens
LCARPRRSPAQEDGKVYINMPGRG

SEQ ID NO: 12 - protein, 112 aa, Artificial Sequence
  aCCR8-1 VL
DIVMTQSPDSLAVSLGERATINCRSSKSLLHSNRNTYLYWYQQKPGQPPKLLIYRMSQLASGVPDRFSGSGSGTDFTLTISSLQAEDVAVYYCMQHLEYPLTFGQGTKLEIK

SEQ ID NO: 13 - protein, 125 aa, Artificial Sequence
  aCCR8-1 VH
EVQLVESGGALVKPGGSLRLSCAASGFTFSTYALYWVRQAPGKGLEWVGRIRSKSNNYATYYADSVKDRFTISRDDSKNTLYLQMNSLKTEDTAVYYCTRARFYYSDYGYAMDYWGQGTLVTVSS

SEQ ID NO: 14 - protein, 112 aa, Artificial Sequence
  aCCR8-2 VL
EIVLTQSPGTLSLSPGERATLSCRSSKSLLHSNGNTYLYWYQQKPGQAPRLLIYRVSNLASGIPDRFSGSGSGTDFTLTISRLEPEDFAVYYCMQHLEYPFTFGQGTKLEIK

SEQ ID NO: 15 - protein, 123 aa, Artificial Sequence
  aCCR8-2 VH
EVQLVESGGALVKPGGSLRLSCAASGFTFSTYAMYWVRQAPGKGLEWVGRIRSKSNNYATYYADSVKDRFTISRDDSKNTLYLQMNSLKTEDTAVYYCTRGGYGNYRYAMDYWGQGTTVTVSS

SEQ ID NO: 16 - protein, 113 aa, Artificial Sequence
  aCCR8-3 VL
DVVLTQTPLSLPVSLGGQASISCRSSQSLVHSNGNTYLHWYLQKPGQSPKLLIYKVSNRFSGVPDRFSGSGSGTDFTLKISRVEAEDLGVYFCSQSTQVPLTFGAGTKLELKR

SEQ ID NO: 17 - protein, 117 aa, Artificial Sequence
  aCCR8-3 VH
QVQLKQSGPSLVQPSQSLSITCTVSGFSLTAYGVHWIRQSPGKGQEWLGVIWRGGSTDYNAAFMSRLTITKDNSKSQVFFKMNSLQADDTAIYYCAKKGGSYAMDYWGQGTSVTVSS

SEQ ID NO: 18 - protein, 114 aa, Artificial Sequence
  aCCR8-4 VL
DIVMTQAAPSVPVTPGESVSISCRSSKSLLHSNGNTYLYWFLQRPGQSPQLLIYRMSNLASGVPDRFSGSGSGTAFTLRISRVEAEDVGVYYCMQHLEYPFTFGSGTKLEIKRA

SEQ ID NO: 19 - protein, 121 aa, Artificial Sequence
  aCCR8-4 VH
EVQLVETGGGLVQPKGSLKLSCAASGFTFNTNAMNWVRQAPGKGLEWVARIRSKSNNYATYYADSVKDRFTISRDDSQSMLYLQMNNLKTEDTAMYYCVREIRPLGDFDVWGAGTTVTVSS

SEQ ID NO: 20 - protein, 115 aa, Artificial Sequence
  aCCR8-5 VL
EIVMTQAVPSVPVTPGESVSISCRSSKSLLHSNGNTYLYWFLQRPGQSPQLLIYRMSNLASGVPDRFSGSGSGTAFTLRISRVEAEDVGVYYCMQHLEYPFTFGSGTKLEIKRAD

SEQ ID NO: 21 - protein, 121 aa, Artificial Sequence
  aCCR8-5 VH
EVQLVETGGGLVQPKGSLKLSCAASGFTFNTNAMNWVRQTPGKGLEWVARIRSKSNNYATYYADSVKDRFTISRDDSQSMLYLQMNNLKTEDTAVYYCVREIRPLGDFDVWGAGTTVTVSS

SEQ ID NO: 22 - protein, 109 aa, Artificial Sequence
  aCCR8-6 VL
ETTVTQSPASLSMAIGEKVTIRCITSTDIDDDMNWYQQKPGEPPKLLISEGNTLRPGVPSRFSSSGYGTDFVFTIENMLSEDVADYYCLQSDNLPYTFGGGTKLEIKRA

SEQ ID NO: 23 - protein, 123 aa, Artificial Sequence
  aCCR8-6 VH
EVQLVESGGGLVQPKGSLKLSCAASGFTFNAYAMNWVRQAPGKGLEWIARIRSKSNNYATYYADSVKDRFTISRDDSQSMLYLQMNNLKTEDTAMYYCVRHKFGRNYYAMDYWGQGTSVTVSS

SEQ ID NO: 24 - protein, 16 aa, Artificial Sequence
  aCCR8-1 VL CDR1
RSSKSLLHSNRNTYLY

SEQ ID NO: 25 - protein, 7 aa, Artificial Sequence
  aCCR8-1 VL CDR2
RMSQLAS

SEQ ID NO: 26 - protein, 9 aa, Artificial Sequence
  aCCR8-1 VL CDR3
MQHLEYPLT

SEQ ID NO: 27 - protein, 5 aa, Artificial Sequence
  aCCR8-1 VH CDR1
TYALY

SEQ ID NO: 28 - protein, 19 aa, Artificial Sequence
  aCCR8-1 VH CDR2
RIRSKSNNYATYYADSVKD

SEQ ID NO: 29 - protein, 14 aa, Artificial Sequence
  aCCR8-1 VH CDR3
ARFYYSDYGYAMDY

SEQ ID NO: 30 - protein, 16 aa, Artificial Sequence
  aCCR8-2 VL CDR1
RSSKSLLHSNGNTYLY

SEQ ID NO: 31 - protein, 7 aa, Artificial Sequence
  aCCR8-2 VL CDR2
RVSNLAS

SEQ ID NO: 32 - protein, 9 aa, Artificial Sequence
  aCCR8-2 VL CDR3
MQHLEYPFT

SEQ ID NO: 33 - protein, 5 aa, Artificial Sequence
  aCCR8-2 VH CDR1
TYAMY

SEQ ID NO: 34 - protein, 12 aa, Artificial Sequence
  aCCR8-2 VH CDR3
GGYGNYRYAMDY

SEQ ID NO: 35 - protein, 16 aa, Artificial Sequence
  aCCR8-3 VL CDR1
RSSQSLVHSNGNTYLH

SEQ ID NO: 36 - protein, 7 aa, Artificial Sequence
  aCCR8-3 VL CDR2
KVSNRFS

SEQ ID NO: 37 - protein, 9 aa, Artificial Sequence
  aCCR8-3 VL CDR3
SQSTQVPLT

SEQ ID NO: 38 - protein, 5 aa, Artificial Sequence
  aCCR8-3 VH CDR1
AYGVH

SEQ ID NO: 39 - protein, 16 aa, Artificial Sequence
  aCCR8-3 VH CDR2
VIWRGGSTDYNAAFMS

SEQ ID NO: 40 - protein, 9 aa, Artificial Sequence
  aCCR8-3 VH CDR3
KGGSYAMDY

SEQ ID NO: 41 - protein, 7 aa, Artificial Sequence
  aCCR8-4 VL CDR2
RMSNLAS

SEQ ID NO: 42 - protein, 5 aa, Artificial Sequence
  aCCR8-4 VH CDR1
TNAMN

SEQ ID NO: 43 - protein, 10 aa, Artificial Sequence
  aCCR8-4 VH CDR3
EIRPLGDFDV

SEQ ID NO: 44 - protein, 10 aa, Artificial Sequence
  aCCR8-6 VL CDR1
TSTDIDDDMN

SEQ ID NO: 45 - protein, 7 aa, Artificial Sequence
  aCCR8-6 VL CDR2
EGNTLRP

SEQ ID NO: 46 - protein, 9 aa, Artificial Sequence
  aCCR8-6 VL CDR3
LQSDNLPYT

SEQ ID NO: 47 - protein, 5 aa, Artificial Sequence
  aCCR8-6 VH CDR1
AYAMN

SEQ ID NO: 48 - protein, 12 aa, Artificial Sequence
  aCCR8-6 VH CDR3
HKFGRNYYAMDY

SEQ ID NO: 49 - protein, 355 aa, Homo sapiens
MDYTLDLSVTTVTDYYYPDIFSSPCDAELIQTNGKLLLAVFYCLLFVFSLLGNSLVILVLVVCKKLRSITDVYLLNLALSDLLFVFSFPFQTYYLLDQWVFGTVMCKVVSGFYYIGFYSSMFFITLMSVDRYLAVVHAVYALKVRTIRMGTTLCLAVWLTAIMATIPLLVFYQVASEDGVLQCYSFYNQQTLKWKIFTNFKMNILGLLIPFTIFMFCYIKILHQLKRCQNHNKTKAIRLVLIVVIASLLFWVPFNVVLFLTSLHSMHILDGCSISQQLTYATHVTEIISFTHCCVNPVIYAFVGEKFKKHLSEIFQKSCSQIFNYLGRQMPRESCEKSSSCQQHSSRSSSVDYIL

SEQ ID NO: 50 - DNA, 43 bp, Artificial Sequence
  pUC19-T7 primer
taatacgactcactatagggagaccagtgaattcgagctcggt

SEQ ID NO: 51 - DNA, 19 bp, Artificial Sequence
  pUC19-R1 primer
gccaagcttgcatgcctgc

SEQ ID NO: 52 - DNA, 43 bp, Artificial Sequence
  T7-AMP-F2 primer
taatacgactcactatagggagatgcttaatcagtgaggcacc

SEQ ID NO: 53 - DNA, 20 bp, Artificial Sequence
  AMP-R1 primer
attcaacatttccgtgtcgc

SEQ ID NO: 54 - protein, 111 aa, Artificial Sequence
  aCCR8-7 VL
DIVLTQSPALAVSLGQRATISCRASQSVSISRYNIMHWYQQKPGQQPKLLIYRASNLASGIPARFSGSGSGTDFTLTINPVQADDIATYYCQQSRESPPTFGGGTKLELKR

SEQ ID NO: 55 - protein, 123 aa, Artificial Sequence
  aCCR8-7 VH
EVQLVESDGGLVQPGRSLKLSCAASGFTFSDYYMAWVRQAPTKGLEWVATITYDVYSTYYRDSVKGRFTISRDNAKSTLYLQMDSLRSEDTATYYCARHGGDGYNSGNWFAYWGQGTLVTVSS

SEQ ID NO: 56 - protein, 21 aa, Artificial Sequence
  aCCR8-7 VL CDR1
RATISCRASQSVSISRYNIMH

SEQ ID NO: 57 - protein, 7 aa, Artificial Sequence
  aCCR8-7 VL CDR2
RASNLAS

SEQ ID NO: 58 - protein, 9 aa, Artificial Sequence
  aCCR8-7 VL CDR3
QQSRESPPT

SEQ ID NO: 59 - protein, 5 aa, Artificial Sequence
  aCCR8-7 VH CDR1
DYYMA

SEQ ID NO: 60 - protein, 16 aa, Artificial Sequence
  aCCR8-7 VH CDR2
TITYDVYSTYYRDSVK

SEQ ID NO: 61 - protein, 14 aa, Artificial Sequence
  aCCR8-7 VH CDR3
HGGDGYNSGNWFAY

SEQ ID NO: 62 - DNA, 2855 bp, Artificial Sequence
  aCCR8-2-CAR-12-IRES-Puromycin DNA
gcggccgccaccatggccctccctgtaactgccctgctgcttcctctggctcttttgttgcatgccgcacgacccgaagtgcaactggtggagagtggcggcgcgctcgtgaagcccggaggcagtctgcgcctgagctgtgccgcatcaggctttacattctcaacatacgccatgtactgggtacgacaagccccgggcaaggggttggagtgggttggccgcatccgctccaagtcaaataattatgccacgtactacgcggatagcgtcaaagataggtttacgatttcaagggatgattcaaagaatacgctgtatctgcaaatgaattcccttaaaaccgaggatacagctgtctactactgcactcgaggtggttatggcaactataggtacgcgatggactactggggccaaggcacaaccgttacggtgagtagcggcggtggcggatctggcggaggcgggagcggaggtggcggttccgaaatagtgctcacgcaaagtcctgggacgctgagcctcagtccaggagaacgagctacgttgtcctgccgatcctccaagagtcttcttcattcaaacggcaacacatacctttactggtatcaacagaaacctggtcaggctccacgactgttgatctaccgcgtcagtaacctggctagtggtatacctgatcgatttagcggatcaggttcaggcacagactttacccttactatcagccgcctggaacccgaggactttgctgtttactactgcatgcaacatcttgagtacccttttacattcgggcagggaacaaagctggagatcaaagctaacgcgtcagattataaggacgatgatgataaaactactactccagcgccacgaccaccgaccccagcgcctacaattgcgagccagccgctgtctttgcgcccagaggcttgcaggccagcagctggaggtgcggtacacacgcgcggcctggacttcgcttgtgatatctacatttgggccccgctggccggaacttgtggtgtactcctgctgagcctggttattacgctgtactgtaaacggggacgaaagaaactcttgtacatattcaagcaaccctttatgaggcccgtacagacgacacaggaagaggacggatgcagctgtcggttccccgaggaggaagagggcggttgtgaactcctctgcgctaggcctcgccgaagccctgcacaggaagacggcaaagtatacattaatatgccgggtagaggccgggtcaaattctctaggtcagcagacgcccctgcatatcaacaagggcagaatcagttgtataatgaattgaacctgggccgccgggaagagtacgatgtcctcgataagagaaggggccgcgacccagagatgggaggaaagccacaacgacgaaagaaccctcaggaaggcctttataatgagcttcagaaggacaaaatggcggaggcctattctgaaatcggcatgaaaggcgagcgcaggcggggcaaagggcacgacggcctctaccaaggtctcagtacagcgacaaaggacacgtacgatgcacttcatatgcaagccctcccacctcggtgataaggatccggaattccgccccccccccccccccccctctccctcccccccccctaacgttactggccgaagccgcttggaataaggccggtgtgcgtttgtctatatgttattttccaccatattgccgtcttttggcaatgtgagggcccggaaacctggccctgtcttcttgacgagcattcctaggggtctttcccctctcgccaaaggaatgcaaggtctgttgaatgtcgtgaaggaagcagttcctctggaagcttcttgaagacaaacaacgtctgtagcgaccctttgcaggcagcggaaccccccacctggcgacaggtgcctctgcggccaaaagccacgtgtataagatacacctgcaaaggcggcacaaccccagtgccacgttgtgagttggatagttgtggaaagagtcaaatggctctcctcaagcgtattcaacaaggggctgaaggatgcccagaaggtaccccattgtatgggatctgatctggggcctcggtgcacatgctttacatgtgtttagtcgaggttaaaaaaacgtctaggccccccgaaccacggggacgtggttttcctttgaaaaacacgatgataagcttgccacaacccacaaggagacgaccttccatgaccgagtacaagcccacggtgcgcctcgccacccgcgacgacgtcccccgggccgtacgcaccctcgccgccgcgttcgccgactaccccgccacgcgccacaccgtcgacccggaccgccacatcgagcgggtcaccgagctgcaagaactcttcctcacgcgcgtcgggctcgacatcggcaaggtgtgggtcgcggacgacggcgccgcggtggcggtctggaccacgccggagagcgtcgaagcgggggcggtgttcgccgagatcggcccgcgcatggccgagttgagcggttcccggctggccgcgcagcaacagatggaaggcctcctggcgccgcaccggcccaaggagcccgcgtggttcctggccaccgtcggcgtctcgcccgaccaccagggcaagggtctgggcagcgccgtcgtgctccccggagtggaggcggccgagcgcgccggggtgcccgccttcctggagacctccgcgccccgcaacctccccttctacgagcggctcggcttcaccgtcaccgccgacgtcgaggtgcccgaaggaccgcgcacctggtgcatgacccgcaagcccggtgcctgagcggccgc